European Patent Application EP 4 740 964 A1, published May 13, 2026. Title: 纳米递送系统、其制备方法和用途. Applicant: 陈海燕. Application WO. The sequence listing filed with the application follows.

SEQUENCE LISTING (21 sequences)

SEQ ID NO: 1 - DNA, 558 bp, synthetic construct
  source 1..558: mol_type = other DNA
atgcaccatcatcatcatcattcttctggtctggtgccacgcggttctggtatgaaagaaaccgctgctgctaaattcgaacgccagcacatggacagcccagatctgggtacccaagctaaacctcaaattccgaaagataaatcgaaagtggcaggctatattgaaattccagatgctgatattaaagaaccagtatatccaggaccagcaacacgggaacaattaaatagaggtgtaagctttgcaaaggaaaatgcctcactagatgatcaaaatatttcaattgcaggacacactttcattgaccgtccgaactatcaatttacaaatcttaaagcagccaaaaaaggtagtatggtgtactttaaagttggtaatgaaacacgtaagtataaaatgacaagtataagaaacgttaagcctacagccgtagaagttctagatgaacaaaaaggtaaagataaacaattaacattaattacttgtgatgattacaatgaagagacaggcgtttgggaaacccgtaaaatctttgtagctacagaagtcaaataa

SEQ ID NO: 2 - DNA, 609 bp, synthetic construct
  source 1..609: mol_type = other DNA
atgcctatgggatctctgcagcctctggccacactgtacctgctgggaatgctggtggctagcgtgctggccggcggaggcggttctggcgatatcatcaagctgctgaacgagcaagtgaacaaagaaatgcaatcctccaacctgtacatgagcatgagcagctggtgttacacccacagccttgatggcgccggactgttcctgtttgatcacgccgccgaggaatacgagcacgccaagaagctgatcatcttcctgaacgagaacaatgtgcccgtgcagctgaccagcattagcgccccagagcacaagttcgagggcctgacacaaatctttcagaaggcctacgaacacgagcagcacatctccgagagcatcaacaacatcgtggaccacgccattaagtccaaggatcacgccaccttcaattttctgcagtggtacgtggccgaacagcacgaggaagaagtgctgttcaaggacatcctggacaagattgagctgatcggcaacgagaaccacggcctgtatctggccgaccagtacgtgaagggaatcgccaagagccggaagtccggcagccaccaccaccatcaccactgatga

SEQ ID NO: 3 - DNA, 1455 bp, synthetic construct
  source 1..1455: mol_type = other DNA
atgggatggtcatgtatcatcctttttctagtagcaactgcaaccggtgtacattcccaggttcagctggttcagtctggcgccgaagtgaagaaacctggcagcagcgtgaaggtgtcctgcaaggcctctggctacgccttcagcagctactggatgaactgggtccgacaggcccctggacaaggcttggaatggatgggacagatctggcctggcgacagcgacaccaattacgcccagaaattccagggcagagtgaccatcaccgccgacgagtctacaagcaccgcctacatggaactgagcagcctgagaagcgaggacaccgccgtgtactactgtgccagacgggaaaccaccaccgtgggcagatattactacgccatggactactggggccagggcaccacagtgacagtctcttctgcgtcgaccaagggcccatcggtcttccccctggcaccctcctccaagagcacctctgggggcacagcggccctgggctgcctggtcaaggactacttccccgaacccgtgacggtgtcgtggaactcaggcgccctgaccagcggcgtgcacaccttcccggctgtcctacagtcctcaggactctactccctcagcagcgtggtgaccgtgccctccagcagcttgggcacccagacctacatctgcaacgtgaatcacaagcccagcaacaccaaggtggacaagaaagttgagcccaaatcttgtgacaaaactcacacatgcccaccgtgcccagcacctgaactcctggggggaccgtcagtcttcctcttccccccaaaacccaaggacaccctcatgatctcccggacccctgaggtcacatgcgtggtggtggacgtgagccacgaagaccctgaggtcaagttcaactggtacgtggacggcgtggaggtgcataatgccaagacaaagccgcgggaggagcagtacaacgccacgtaccgtgtggtcagcgtcctcaccgtcctgcaccaggactggctgaatggcaaggagtacaagtgcaaggtctccaacaaagccctcccagcccccatcgcggcaaccatctccaaagccaaagggcagccccgagaaccacaggtgtacaccctgcccccatcccgggatgagctgaccaagaaccaggtcagcctgacctgcctggtcaaaggcttctatcccagcgacatcgccgtggagtgggagagcaatgggcagccggagaacaactacaagaccacgcctcccgtgctggactccgacggctccttcttcctctacagcaagctcaccgtggacaagagcaggtggcagcaggggaacgtcttctcatgctccgtgatgcatgaggctctgcacgcccactacacgcagaagagcctctccctgtctccgggtaaaagcggcggcagcggcctgcctgagaccggaggatga

SEQ ID NO: 4 - DNA, 780 bp, synthetic construct
  source 1..780: mol_type = other DNA
atgggatggtcatgtatcatcctttttctagtagcaactgcaaccggtgtacattcccaggttcagctggttcagtctggcgccgaagtgaagaaacctggcagcagcgtgaaggtgtcctgcaaggcctctggctacgccttcagcagctactggatgaactgggtccgacaggcccctggacaaggcttggaatggatgggacagatctggcctggcgacagcgacaccaattacgcccagaaattccagggcagagtgaccatcaccgccgacgagtctacaagcaccgcctacatggaactgagcagcctgagaagcgaggacaccgccgtgtactactgtgccagacgggaaaccaccaccgtgggcagatattactacgccatggactactggggccagggcaccacagtgacagtctcttctgcgtcgaccaagggcccatcggtcttccccctggcaccctcctccaagagcacctctgggggcacagcggccctgggctgcctggtcaaggactacttccccgaacccgtgacggtgtcgtggaactcaggcgccctgaccagcggcgtgcacaccttcccggctgtcctacagtcctcaggactctactccctcagcagcgtggtgaccgtgccctccagcagcttgggcacccagacctacatctgcaacgtgaatcacaagcccagcaacaccaaggtggacaagaaagttgagcccaaatcttgtgacaaaagcggcggcagcggcctgcctgagaccggaggatga

SEQ ID NO: 5 - DNA, 714 bp, synthetic construct
  source 1..714: mol_type = other DNA
atgggatggtcatgtatcatcctttttctagtagcaactgcaaccggtgtacattcagacatccagctgacccagtctccaagctttctgagcgccagcgtgggcgacagagtgaccatcacatgtaaagccagccagagcgtggactacagcggcgacagctacctgaactggtatcagcagaagcccggcaaggcccctaagctgctgatctacgatgccagcaatctggtgtccggcgtgcccagcagattttctggctctggaagcggcaccgagttcaccctgaccatatctagcctgcagcctgaggacttcgccacctactactgccagcagagcaccgagaatccctggacatttggcggaggcaccaagctggaaatcaagcgtacggtggctgcaccatctgtcttcatcttcccgccatctgatgagcagttgaaatctggaactgcctctgttgtgtgcctgctgaataacttctaccccagagaagccaaagtgcagtggaaggtggacaacgccctgcagagcggaaacagccaggaaagcgtgacagagcaggattccaaggattccacatacagcctgagcagcacactgacactgtccaaggccgactacgagaagcacaaggtgtacgcctgcgaagtgacacaccagggactgtcctcccctgtgacaaagagcttcaacagaggagaatgctga

SEQ ID NO: 6 - DNA, 428 bp, synthetic construct
  source 1..428: mol_type = other DNA
atgggatggtcatgtatcatcctttttctagtagcaactgcaaccggtgtacattcccaggtacaactgcagcagcctggggctgagctggtgaagcctggggcctcagtgaagatgtcctgcaaggcttctggctacacatttaccagttacaatatgcactgggtaaaacagacacctggtcggggcctggaatggattggagctatttatcccggaaatggtgatacttcctacaatcagaagttcaaaggcaaggccacattgactgcagacaaatcctccagcacagcctacatgcagctcagcagcctgacatctgaggactctgcggtctattactgtgcaagatcgacttactacggcggtgactggtacttcaatgtctggggcgcagggaccacggtcaccgtctctgcagcgtcgac

SEQ ID NO: 7 - DNA, 381 bp, synthetic construct
  source 1..381: mol_type = other DNA
atgggatggtcatgtatcatcctttttctagtagcaactgcaaccggtgtacattcacaaattgttctctcccagtctccagcaatcctgtctgcatctccaggggagaaggtcacaatgacttgcagggccagctcaagtgtaagttacatccactggttccagcagaagccaggctcctcccccaaaccctggatttatgccacatccaacctggcttctggagtccctgttcgcttcagtggcagtgggtctgggacttcttactctctcacaatcagcagagtggaggctgaagatgctgccacttattactgccagcagtggactagtaacccacccacgttcggaggggggaccaagctggaaatcaaacgtacg

SEQ ID NO: 8 - DNA, 428 bp, synthetic construct
  source 1..428: mol_type = other DNA
atgggatggtcatgtatcatcctttttctagtagcaactgcaaccggtgtacattccgaagtgcagctggttcagtctggcgccgaagtgaagaaacctggcgcctctgtgaaggtgtcctgcaaggccagcggctaccgcttcaccaactactggatacactgggtccgacaggcccctggacaaggactggaatggatcggcggcatcaaccccggcaacaactacgccacctaccggcggaagtttcagggcagagtgaccatgaccgccgacaccagcacaagcaccgtgtacatggaactgagcagcctgagaagcgaggacaccgccgtgtactactgcaccagagaaggctacggcaactacggcgcttggtttgcctattggggccagggcacactggtcaccgttagctctgcgtcgac

SEQ ID NO: 9 - DNA, 399 bp, synthetic construct
  source 1..399: mol_type = other DNA
atgggatggtcatgtatcatcctttttctagtagcaactgcaaccggtgtacattcagacgtgcaagtgacacagagcccttctagcctgtctgccagcgtgggcgacagagtgaccatcacctgtagaagcagccagagcctggccaacagctacggcaataccttcctgagctggtatctgcacaagcccggaaaggctccccagctgctgatctacggcatcagcaacagattcagcggcgtgcccgataggtttagcggctctggaagcggcaccgacttcaccctgaccatatctagcctgcagcctgaggacttcgccacctactactgtctgcaaggcacccaccagccttacacctttggccagggcaccaaggtggaaatcaagcgtacg

SEQ ID NO: 10 - protein, 185 aa, synthetic construct
MHHHHHHSSGLVPRGSGMKETAAAKFERQHMDSPDLGTQAKPQIPKDKSKVAGYIEIPDADIKEPVYPGPATREQLNRGVSFAKENASLDDQNISIAGHTFIDRPNYQFTNLKAAKKGSMVYFKVGNETRKYKMTSIRNVKPTAVEVLDEQKGKDKQLTLITCDDYNEETGVWETRKIFVATEVK

SEQ ID NO: 11 - protein, 201 aa, synthetic construct
MPMGSLQPLATLYLLGMLVASVLAGGGGSGDIIKLLNEQVNKEMQSSNLYMSMSSWCYTHSLDGAGLFLFDHAAEEYEHAKKLIIFLNENNVPVQLTSISAPEHKFEGLTQIFQKAYEHEQHISESINNIVDHAIKSKDHATFNFLQWYVAEQHEEEVLFKDILDKIELIGNENHGLYLADQYVKGIAKSRKSGSHHHHHH

SEQ ID NO: 12 - protein, 484 aa, synthetic construct
MGWSCIILFLVATATGVHSQVQLVQSGAEVKKPGSSVKVSCKASGYAFSSYWMNWVRQAPGQGLEWMGQIWPGDSDTNYAQKFQGRVTITADESTSTAYMELSSLRSEDTAVYYCARRETTTVGRYYYAMDYWGQGTTVTVSSASTKGPSVFPLAPSSKSTSGGTAALGCLVKDYFPEPVTVSWNSGALTSGVHTFPAVLQSSGLYSLSSVVTVPSSSLGTQTYICNVNHKPSNTKVDKKVEPKSCDKTHTCPPCPAPELLGGPSVFLFPPKPKDTLMISRTPEVTCVVVDVSHEDPEVKFNWYVDGVEVHNAKTKPREEQYNATYRVVSVLTVLHQDWLNGKEYKCKVSNKALPAPIAATISKAKGQPREPQVYTLPPSRDELTKNQVSLTCLVKGFYPSDIAVEWESNGQPENNYKTTPPVLDSDGSFFLYSKLTVDKSRWQQGNVFSCSVMHEALHAHYTQKSLSLSPGKSGGSGLPETGG

SEQ ID NO: 13 - protein, 259 aa, synthetic construct
MGWSCIILFLVATATGVHSQVQLVQSGAEVKKPGSSVKVSCKASGYAFSSYWMNWVRQAPGQGLEWMGQIWPGDSDTNYAQKFQGRVTITADESTSTAYMELSSLRSEDTAVYYCARRETTTVGRYYYAMDYWGQGTTVTVSSASTKGPSVFPLAPSSKSTSGGTAALGCLVKDYFPEPVTVSWNSGALTSGVHTFPAVLQSSGLYSLSSVVTVPSSSLGTQTYICNVNHKPSNTKVDKKVEPKSCDKSGGSGLPETGG

SEQ ID NO: 14 - protein, 237 aa, synthetic construct
MGWSCIILFLVATATGVHSDIQLTQSPSFLSASVGDRVTITCKASQSVDYSGDSYLNWYQQKPGKAPKLLIYDASNLVSGVPSRFSGSGSGTEFTLTISSLQPEDFATYYCQQSTENPWTFGGGTKLEIKRTVAAPSVFIFPPSDEQLKSGTASVVCLLNNFYPREAKVQWKVDNALQSGNSQESVTEQDSKDSTYSLSSTLTLSKADYEKHKVYACEVTHQGLSSPVTKSFNRGEC

SEQ ID NO: 15 - protein, 481 aa, synthetic construct
MGWSCIILFLVATATGVHSQVQLQQPGAELVKPGASVKMSCKASGYTFTSYNMHWVKQTPGRGLEWIGAIYPGNGDTSYNQKFKGKATLTADKSSSTAYMQLSSLTSEDSAVYYCARSTYYGGDWYFNVWGAGTTVTVSAASTKGPSVFPLAPSSKSTSGGTAALGCLVKDYFPEPVTVSWNSGALTSGVHTFPAVLQSSGLYSLSSVVTVPSSSLGTQTYICNVNHKPSNTKVDKKVEPKSCDKTHTCPPCPAPELLGGPSVFLFPPKPKDTLMISRTPEVTCVVVDVSHEDPEVKFNWYVDGVEVHNAKTKPREEQYNATYRVVSVLTVLHQDWLNGKEYKCKVSNKALPAPIAATISKAKGQPREPQVYTLPPSRDELTKNQVSLTCLVKGFYPSDIAVEWESNGQPENNYKTTPPVLDSDGSFFLYSKLTVDKSRWQQGNVFSCSVMHEALHAHYTQKSLSLSPGKSGGSGLPETGG

SEQ ID NO: 16 - protein, 232 aa, synthetic construct
MGWSCIILFLVATATGVHSQIVLSQSPAILSASPGEKVTMTCRASSSVSYIHWFQQKPGSSPKPWIYATSNLASGVPVRFSGSGSGTSYSLTISRVEAEDAATYYCQQWTSNPPTFGGGTKLEIKRTVAAPSVFIFPPSDEQLKSGTASVVCLLNNFYPREAKVQWKVDNALQSGNSQESVTEQDSKDSTYSLSSTLTLSKADYEKHKVYACEVTHQGLSSPVTKSFNRGEC

SEQ ID NO: 17 - protein, 481 aa, synthetic construct
MGWSCIILFLVATATGVHSEVQLVQSGAEVKKPGASVKVSCKASGYRFTNYWIHWVRQAPGQGLEWIGGINPGNNYATYRRKFQGRVTMTADTSTSTVYMELSSLRSEDTAVYYCTREGYGNYGAWFAYWGQGTLVTVSSASTKGPSVFPLAPSSKSTSGGTAALGCLVKDYFPEPVTVSWNSGALTSGVHTFPAVLQSSGLYSLSSVVTVPSSSLGTQTYICNVNHKPSNTKVDKKVEPKSCDKTHTCPPCPAPELLGGPSVFLFPPKPKDTLMISRTPEVTCVVVDVSHEDPEVKFNWYVDGVEVHNAKTKPREEQYNATYRVVSVLTVLHQDWLNGKEYKCKVSNKALPAPIAATISKAKGQPREPQVYTLPPSRDELTKNQVSLTCLVKGFYPSDIAVEWESNGQPENNYKTTPPVLDSDGSFFLYSKLTVDKSRWQQGNVFSCSVMHEALHAHYTQKSLSLSPGKSGGSGLPETGG

SEQ ID NO: 18 - protein, 238 aa, synthetic construct
MGWSCIILFLVATATGVHSDVQVTQSPSSLSASVGDRVTITCRSSQSLANSYGNTFLSWYLHKPGKAPQLLIYGISNRFSGVPDRFSGSGSGTDFTLTISSLQPEDFATYYCLQGTHQPYTFGQGTKVEIKRTVAAPSVFIFPPSDEQLKSGTASVVCLLNNFYPREAKVQWKVDNALQSGNSQESVTEQDSKDSTYSLSSTLTLSKADYEKHKVYACEVTHQGLSSPVTKSFNRGEC

SEQ ID NO: 19 - protein, 8 aa, synthetic construct
LPXTGGGG

SEQ ID NO: 20 - protein, 4 aa, synthetic construct
GGGG

SEQ ID NO: 21 - protein, 6 aa, synthetic construct
LPXTGG